European Patent Application EP 4 159 764 A1, published April 5, 2023. Title: Anti-PDL1×EGFR bispecific antibody. Applicant: ZEDA BIOPHARMACEUTICALS, INC. The sequence listing filed with the application follows.

SEQUENCE LISTING (29 sequences)

SEQ ID NO: 1 - protein, 11 aa, Artificial Sequence
  Amino acid sequence of light chain complementary determinant L-CDR1 of anti-PD-L1 monoclonal antibody
RASQSIGTTIH

SEQ ID NO: 2 - protein, 7 aa, Artificial Sequence
  Amino acid sequence of light chain complementary determinant L-CDR2 of anti-PD-L1 monoclonal antibody
YASQSFS

SEQ ID NO: 3 - protein, 9 aa, Artificial Sequence
  Amino acid sequence of light chain complementary determinant L-CDR3 of anti-PD-L1 monoclonal antibody
QQSNSWPLT

SEQ ID NO: 4 - protein, 5 aa, Artificial Sequence
  Amino acid sequence of heavy chain complementary determinant H-CDR1 of anti-PD-L1 monoclonal antibody
SYGVH

SEQ ID NO: 5 - protein, 16 aa, Artificial Sequence
  Amino acid sequence of heavy chain complementary determinant H-CDR2 of anti-PD-L1 monoclonal antibody
LIWSGGGTDYNPSLKS

SEQ ID NO: 6 - protein, 9 aa, Artificial Sequence
  Amino acid sequence of heavy chain complementary determinant H-CDR3 of anti-PD-L1 monoclonal antibody
QLGLRAMDY

SEQ ID NO: 7 - protein, 10 aa, Artificial Sequence
  Amino acid sequence of the heavy chain complementary determinant H-CDR1 of anti-EGFR monoclonal antibody
GFSLTNYGVH

SEQ ID NO: 8 - protein, 16 aa, Artificial Sequence
  Amino acid sequence of the heavy chain complementary determinant H-CDR2 of anti-EGFR monoclonal antibody
VIWSGGNTDYNTPFTS

SEQ ID NO: 9 - protein, 11 aa, Artificial Sequence
  Amino acid sequence of the heavy chain complementary determinant H-CDR3 of anti-EGFR monoclonal antibody
ALTYYDYEFAY

SEQ ID NO: 10 - protein, 11 aa, Artificial Sequence
  Amino acid sequence of the light chain complementary determinant L-CDR1 of anti-EGFR monoclonal antibody
RASQSIGTNIH

SEQ ID NO: 11 - protein, 7 aa, Artificial Sequence
  Amino acid sequence of the light chain complementary determinant L-CDR2 of anti-EGFR monoclonal antibody
YASESIS

SEQ ID NO: 12 - protein, 9 aa, Artificial Sequence
  Amino acid sequence of the light chain complementary determinant L-CDR3 of anti-EGFR monoclonal antibody
QQNNNWPTT

SEQ ID NO: 13 - protein, 107 aa, Artificial Sequence
  Amino acid sequence of the light chain variable region of anti-PD-L1 monoclonal antibody
EIVLTQSPDFLSVTPKEKVTITCRASQSIGTTIHWYQQKPDQSPKLLIKYASQSFSGVPSRFSGSGSGTDFTLTINSVEAEDAATYYCQQSNSWPLTFGAGTKLEIK

SEQ ID NO: 14 - protein, 117 aa, Artificial Sequence
  Amino acid sequence of the heavy chain variable region of anti-PD-L1 monoclonal antibody
QVQLQQSGGGLVKPSQSLSLTCTVSGFSLTSYGVHWVRQPPGKGLEWIGLIWSGGGTDYNPSLKSRLTISRDTSKNQVSFKISSLTAADTAVYYCARQLGLRAMDYWGQGTSVTVSS

SEQ ID NO: 15 - protein, 119 aa, Artificial Sequence
  Amino acid sequence of the heavy chain variable region of anti-EGFR monoclonal antibody
QVQLKQSGPGLVQPSQSLSITCTVSGFSLTNYGVHWVRQSPGKGLEWLGVIWSGGNTDYNTPFTSRLSINKDNSKSQVFFKMNSLQSNDTAIYYCARALTYYDYEFAYWGQGTLVTVSA

SEQ ID NO: 16 - protein, 107 aa, Artificial Sequence
  Amino acid sequence of light chain variable region of anti-EGFR monoclonal antibody
DILLTQSPVILSVSPGERVSFSCRASQSIGTNIHWYQQRTNGSPRLLIKYASESISGIPSRFSGSGSGTDFTLSINSVESEDIADYYCQQNNNWPTTFGAGTKLELK

SEQ ID NO: 17 - protein, 708 aa, Artificial Sequence
  Amino acid sequence of anti-PDL1×EGFR BsAb1 polypeptide chain
EIVLTQSPDFLSVTPKEKVTITCRASQSIGTTIHWYQQKPDQSPKLLIKYASQSFSGVPSRFSGSGSGTDFTLTINSVEAEDAATYYCQQSNSWPLTFGAGTKLEIKGGGGSGGGGSGGGGSGGGGSQVQLQQSGGGLVKPSQSLSLTCTVSGFSLTSYGVHWVRQPPGKGLEWIGLIWSGGGTDYNPSLKSRLTISRDTSKNQVSFKISSLTAADTAVYYCARQLGLRAMDYWGQGTSVTVSSGGGGSGGGGSGGGGSQVQLKQSGPGLVQPSQSLSITCTVSGFSLTNYGVHWVRQSPGKGLEWLGVIWSGGNTDYNTPFTSRLSINKDNSKSQVFFKMNSLQSNDTAIYYCARALTYYDYEFAYWGQGTLVTVSAASTKGPSVFPLAPSSKSTSGGTAALGCLVKDYFPEPVTVSWNSGALTSGVHTFPAVLQSSGLYSLSSVVTVPSSSLGTQTYICNVNHKPSNTKVDKKVEPKSCDKTHTCPPCPAPELLGGPSVFLFPPKPKDTLMISRTPEVTCVVVDVSHEDPEVKFNWYVDGVEVHNAKTKPREEQYNSTYRVVSVLTVLHQDWLNGKEYKCKVSNKALPAPIEKTISKAKGQPREPQVYTLPPSREEMTKNQVSLTCLVKGFYPSDIAVEWESNGQPENNYKTTPPVLDSDGSFFLYSKLTVDKSRWQQGNVFSCSVMHEALHNHYTQKSLSLSPGK

SEQ ID NO: 18 - protein, 713 aa, Artificial Sequence
  Amino acid sequence of anti-PDL1×EGFR BsAb2 polypeptide chain
EIVLTQSPDFLSVTPKEKVTITCRASQSIGTTIHWYQQKPDQSPKLLIKYASQSFSGVPSRFSGSGSGTDFTLTINSVEAEDAATYYCQQSNSWPLTFGAGTKLEIKGGGGSGGGGSGGGGSGGGGSGGGGSQVQLQQSGGGLVKPSQSLSLTCTVSGFSLTSYGVHWVRQPPGKGLEWIGLIWSGGGTDYNPSLKSRLTISRDTSKNQVSFKISSLTAADTAVYYCARQLGLRAMDYWGQGTSVTVSSGGGGSGGGGSGGGGSQVQLKQSGPGLVQPSQSLSITCTVSGFSLTNYGVHWVRQSPGKGLEWLGVIWSGGNTDYNTPFTSRLSINKDNSKSQVFFKMNSLQSNDTAIYYCARALTYYDYEFAYWGQGTLVTVSAASTKGPSVFPLAPSSKSTSGGTAALGCLVKDYFPEPVTVSWNSGALTSGVHTFPAVLQSSGLYSLSSVVTVPSSSLGTQTYICNVNHKPSNTKVDKKVEPKSCDKTHTCPPCPAPELLGGPSVFLFPPKPKDTLMISRTPEVTCVVVDVSHEDPEVKFNWYVDGVEVHNAKTKPREEQYNSTYRVVSVLTVLHQDWLNGKEYKCKVSNKALPAPIEKTISKAKGQPREPQVYTLPPSREEMTKNQVSLTCLVKGFYPSDIAVEWESNGQPENNYKTTPPVLDSDGSFFLYSKLTVDKSRWQQGNVFSCSVMHEALHNHYTQKSLSLSPGK

SEQ ID NO: 19 - protein, 214 aa, Artificial Sequence
  The light chain amino acid sequence of anti-EGFR monoclonal antibody
DILLTQSPVILSVSPGERVSFSCRASQSIGTNIHWYQQRTNGSPRLLIKYASESISGIPSRFSGSGSGTDFTLSINSVESEDIADYYCQQNNNWPTTFGAGTKLELKRTVAAPSVFIFPPSDEQLKSGTASVVCLLNNFYPREAKVQWKVDNALQSGNSQESVTEQDSKDSTYSLSSTLTLSKADYEKHKVYACEVTHQGLSSPVTKSFNRGEC

SEQ ID NO: 20 - protein, 449 aa, Artificial Sequence
  The heavy chain amino acid sequence of anti-EGFR monoclonal antibody
QVQLKQSGPGLVQPSQSLSITCTVSGFSLTNYGVHWVRQSPGKGLEWLGVIWSGGNTDYNTPFTSRLSINKDNSKSQVFFKMNSLQSNDTAIYYCARALTYYDYEFAYWGQGTLVTVSAASTKGPSVFPLAPSSKSTSGGTAALGCLVKDYFPEPVTVSWNSGALTSGVHTFPAVLQSSGLYSLSSVVTVPSSSLGTQTYICNVNHKPSNTKVDKKVEPKSCDKTHTCPPCPAPELLGGPSVFLFPPKPKDTLMISRTPEVTCVVVDVSHEDPEVKFNWYVDGVEVHNAKTKPREEQYNSTYRVVSVLTVLHQDWLNGKEYKCKVSNKALPAPIEKTISKAKGQPREPQVYTLPPSREEMTKNQVSLTCLVKGFYPSDIAVEWESNGQPENNYKTTPPVLDSDGSFFLYSKLTVDKSRWQQGNVFSCSVMHEALHNHYTQKSLSLSPGK

SEQ ID NO: 21 - protein, 447 aa, Artificial Sequence
  The heavy chain amino acid sequence of anti-PD-L1 monoclonal antibody
QVQLQQSGGGLVKPSQSLSLTCTVSGFSLTSYGVHWVRQPPGKGLEWIGLIWSGGGTDYNPSLKSRLTISRDTSKNQVSFKISSLTAADTAVYYCARQLGLRAMDYWGQGTSVTVSSASTKGPSVFPLAPSSKSTSGGTAALGCLVKDYFPEPVTVSWNSGALTSGVHTFPAVLQSSGLYSLSSVVTVPSSSLGTQTYICNVNHKPSNTKVDKKVEPKSCDKTHTCPPCPAPELLGGPSVFLFPPKPKDTLMISRTPEVTCVVVDVSHEDPEVKFNWYVDGVEVHNAKTKPREEQYNSTYRVVSVLTVLHQDWLNGKEYKCKVSNKALPAPIEKTISKAKGQPREPQVYTLPPSREEMTKNQVSLTCLVKGFYPSDIAVEWESNGQPENNYKTTPPVLDSDGSFFLYSKLTVDKSRWQQGNVFSCSVMHEALHNHYTQKSLSLSPGK

SEQ ID NO: 22 - protein, 214 aa, Artificial Sequence
  The light chain amino acid sequence of anti-PD-L1 monoclonal antibody
EIVLTQSPDFLSVTPKEKVTITCRASQSIGTTIHWYQQKPDQSPKLLIKYASQSFSGVPSRFSGSGSGTDFTLTINSVEAEDAATYYCQQSNSWPLTFGAGTKLEIKRTVAAPSVFIFPPSDEQLKSGTASVVCLLNNFYPREAKVQWKVDNALQSGNSQESVTEQDSKDSTYSLSSTLTLSKADYEKHKVYACEVTHQGLSSPVTKSFNRGEC

SEQ ID NO: 23 - protein, 708 aa, Artificial Sequence
  Amino acid sequence of anti-PDL1×EGFR BsAb rev1 polypeptide chain
QVQLKQSGPGLVQPSQSLSITCTVSGFSLTNYGVHWVRQSPGKGLEWLGVIWSGGNTDYNTPFTSRLSINKDNSKSQVFFKMNSLQSNDTAIYYCARALTYYDYEFAYWGQGTLVTVSAASTKGPSVFPLAPSSKSTSGGTAALGCLVKDYFPEPVTVSWNSGALTSGVHTFPAVLQSSGLYSLSSVVTVPSSSLGTQTYICNVNHKPSNTKVDKKVEPKSCDKTHTCPPCPAPELLGGPSVFLFPPKPKDTLMISRTPEVTCVVVDVSHEDPEVKFNWYVDGVEVHNAKTKPREEQYNSTYRVVSVLTVLHQDWLNGKEYKCKVSNKALPAPIEKTISKAKGQPREPQVYTLPPSREEMTKNQVSLTCLVKGFYPSDIAVEWESNGQPENNYKTTPPVLDSDGSFFLYSKLTVDKSRWQQGNVFSCSVMHEALHNHYTQKSLSLSPGKGGGGSGGGGSGGGGSEIVLTQSPDFLSVTPKEKVTITCRASQSIGTTIHWYQQKPDQSPKLLIKYASQSFSGVPSRFSGSGSGTDFTLTINSVEAEDAATYYCQQSNSWPLTFGAGTKLEIKGGGGSGGGGSGGGGSGGGGSQVQLQQSGGGLVKPSQSLSLTCTVSGFSLTSYGVHWVRQPPGKGLEWIGLIWSGGGTDYNPSLKSRLTISRDTSKNQVSFKISSLTAADTAVYYCARQLGLRAMDYWGQGTSVTVSS

SEQ ID NO: 24 - protein, 708 aa, Artificial Sequence
  Amino acid sequence of anti-PDL1×EGFR BsAb rev2 polypeptide chain
QVQLKQSGPGLVQPSQSLSITCTVSGFSLTNYGVHWVRQSPGKGLEWLGVIWSGGNTDYNTPFTSRLSINKDNSKSQVFFKMNSLQSNDTAIYYCARALTYYDYEFAYWGQGTLVTVSAASTKGPSVFPLAPSSKSTSGGTAALGCLVKDYFPEPVTVSWNSGALTSGVHTFPAVLQSSGLYSLSSVVTVPSSSLGTQTYICNVNHKPSNTKVDKKVEPKSCDKTHTCPPCPAPELLGGPSVFLFPPKPKDTLMISRTPEVTCVVVDVSHEDPEVKFNWYVDGVEVHNAKTKPREEQYNSTYRVVSVLTVLHQDWLNGKEYKCKVSNKALPAPIEKTISKAKGQPREPQVYTLPPSREEMTKNQVSLTCLVKGFYPSDIAVEWESNGQPENNYKTTPPVLDSDGSFFLYSKLTVDKSRWQQGNVFSCSVMHEALHNHYTQKSLSLSPGKGGGGSGGGGSGGGGSQVQLQQSGGGLVKPSQSLSLTCTVSGFSLTSYGVHWVRQPPGKGLEWIGLIWSGGGTDYNPSLKSRLTISRDTSKNQVSFKISSLTAADTAVYYCARQLGLRAMDYWGQGTSVTVSSGGGGSGGGGSGGGGSGGGGSEIVLTQSPDFLSVTPKEKVTITCRASQSIGTTIHWYQQKPDQSPKLLIKYASQSFSGVPSRFSGSGSGTDFTLTINSVEAEDAATYYCQQSNSWPLTFGAGTKLEIK

SEQ ID NO: 25 - protein, 708 aa, Artificial Sequence
  Amino acid sequence of anti-PDL1×EGFR BsAb rev3 polypeptide chain
QVQLQQSGGGLVKPSQSLSLTCTVSGFSLTSYGVHWVRQPPGKGLEWIGLIWSGGGTDYNPSLKSRLTISRDTSKNQVSFKISSLTAADTAVYYCARQLGLRAMDYWGQGTSVTVSSGGGGSGGGGSGGGGSGGGGSEIVLTQSPDFLSVTPKEKVTITCRASQSIGTTIHWYQQKPDQSPKLLIKYASQSFSGVPSRFSGSGSGTDFTLTINSVEAEDAATYYCQQSNSWPLTFGAGTKLEIKGGGGSGGGGSGGGGSQVQLKQSGPGLVQPSQSLSITCTVSGFSLTNYGVHWVRQSPGKGLEWLGVIWSGGNTDYNTPFTSRLSINKDNSKSQVFFKMNSLQSNDTAIYYCARALTYYDYEFAYWGQGTLVTVSAASTKGPSVFPLAPSSKSTSGGTAALGCLVKDYFPEPVTVSWNSGALTSGVHTFPAVLQSSGLYSLSSVVTVPSSSLGTQTYICNVNHKPSNTKVDKKVEPKSCDKTHTCPPCPAPELLGGPSVFLFPPKPKDTLMISRTPEVTCVVVDVSHEDPEVKFNWYVDGVEVHNAKTKPREEQYNSTYRVVSVLTVLHQDWLNGKEYKCKVSNKALPAPIEKTISKAKGQPREPQVYTLPPSREEMTKNQVSLTCLVKGFYPSDIAVEWESNGQPENNYKTTPPVLDSDGSFFLYSKLTVDKSRWQQGNVFSCSVMHEALHNHYTQKSLSLSPGK

SEQ ID NO: 26 - protein, 708 aa, Artificial Sequence
  Amino acid sequence of anti-PDL1×EGFR BsAb rev5 polypeptide chain
QVQLQQSGGGLVKPSQSLSLTCTVSGFSLTSYGVHWVRQPPGKGLEWIGLIWSGGGTDYNPSLKSRLTISRDTSKNQVSFKISSLTAADTAVYYCARQLGLRAMDYWGQGTSVTVSSASTKGPSVFPLAPSSKSTSGGTAALGCLVKDYFPEPVTVSWNSGALTSGVHTFPAVLQSSGLYSLSSVVTVPSSSLGTQTYICNVNHKPSNTKVDKKVEPKSCDKTHTCPPCPAPELLGGPSVFLFPPKPKDTLMISRTPEVTCVVVDVSHEDPEVKFNWYVDGVEVHNAKTKPREEQYNSTYRVVSVLTVLHQDWLNGKEYKCKVSNKALPAPIEKTISKAKGQPREPQVYTLPPSREEMTKNQVSLTCLVKGFYPSDIAVEWESNGQPENNYKTTPPVLDSDGSFFLYSKLTVDKSRWQQGNVFSCSVMHEALHNHYTQKSLSLSPGKGGGGSGGGGSGGGGSDILLTQSPVILSVSPGERVSFSCRASQSIGTNIHWYQQRTNGSPRLLIKYASESISGIPSRFSGSGSGTDFTLSINSVESEDIADYYCQQNNNWPTTFGAGTKLELKGGGGSGGGGSGGGGSGGGGSQVQLKQSGPGLVQPSQSLSITCTVSGFSLTNYGVHWVRQSPGKGLEWLGVIWSGGNTDYNTPFTSRLSINKDNSKSQVFFKMNSLQSNDTAIYYCARALTYYDYEFAYWGQGTLVTVSA

SEQ ID NO: 27 - protein, 708 aa, Artificial Sequence
  Amino acid sequence of anti-PDL1×EGFR BsAb rev6 polypeptide chain
QVQLQQSGGGLVKPSQSLSLTCTVSGFSLTSYGVHWVRQPPGKGLEWIGLIWSGGGTDYNPSLKSRLTISRDTSKNQVSFKISSLTAADTAVYYCARQLGLRAMDYWGQGTSVTVSSASTKGPSVFPLAPSSKSTSGGTAALGCLVKDYFPEPVTVSWNSGALTSGVHTFPAVLQSSGLYSLSSVVTVPSSSLGTQTYICNVNHKPSNTKVDKKVEPKSCDKTHTCPPCPAPELLGGPSVFLFPPKPKDTLMISRTPEVTCVVVDVSHEDPEVKFNWYVDGVEVHNAKTKPREEQYNSTYRVVSVLTVLHQDWLNGKEYKCKVSNKALPAPIEKTISKAKGQPREPQVYTLPPSREEMTKNQVSLTCLVKGFYPSDIAVEWESNGQPENNYKTTPPVLDSDGSFFLYSKLTVDKSRWQQGNVFSCSVMHEALHNHYTQKSLSLSPGKGGGGSGGGGSGGGGSQVQLKQSGPGLVQPSQSLSITCTVSGFSLTNYGVHWVRQSPGKGLEWLGVIWSGGNTDYNTPFTSRLSINKDNSKSQVFFKMNSLQSNDTAIYYCARALTYYDYEFAYWGQGTLVTVSAGGGGSGGGGSGGGGSGGGGSDILLTQSPVILSVSPGERVSFSCRASQSIGTNIHWYQQRTNGSPRLLIKYASESISGIPSRFSGSGSGTDFTLSINSVESEDIADYYCQQNNNWPTTFGAGTKLELK

SEQ ID NO: 28 - protein, 708 aa, Artificial Sequence
  Amino acid sequence of anti-PDL1×EGFR BsAb rev7 polypeptide chain
QVQLKQSGPGLVQPSQSLSITCTVSGFSLTNYGVHWVRQSPGKGLEWLGVIWSGGNTDYNTPFTSRLSINKDNSKSQVFFKMNSLQSNDTAIYYCARALTYYDYEFAYWGQGTLVTVSAGGGGSGGGGSGGGGSGGGGSDILLTQSPVILSVSPGERVSFSCRASQSIGTNIHWYQQRTNGSPRLLIKYASESISGIPSRFSGSGSGTDFTLSINSVESEDIADYYCQQNNNWPTTFGAGTKLELKGGGGSGGGGSGGGGSQVQLQQSGGGLVKPSQSLSLTCTVSGFSLTSYGVHWVRQPPGKGLEWIGLIWSGGGTDYNPSLKSRLTISRDTSKNQVSFKISSLTAADTAVYYCARQLGLRAMDYWGQGTSVTVSSASTKGPSVFPLAPSSKSTSGGTAALGCLVKDYFPEPVTVSWNSGALTSGVHTFPAVLQSSGLYSLSSVVTVPSSSLGTQTYICNVNHKPSNTKVDKKVEPKSCDKTHTCPPCPAPELLGGPSVFLFPPKPKDTLMISRTPEVTCVVVDVSHEDPEVKFNWYVDGVEVHNAKTKPREEQYNSTYRVVSVLTVLHQDWLNGKEYKCKVSNKALPAPIEKTISKAKGQPREPQVYTLPPSREEMTKNQVSLTCLVKGFYPSDIAVEWESNGQPENNYKTTPPVLDSDGSFFLYSKLTVDKSRWQQGNVFSCSVMHEALHNHYTQKSLSLSPGK

SEQ ID NO: 29 - protein, 708 aa, Artificial Sequence
  Amino acid sequence of anti-PDL1×EGFR BsAb rev8 polypeptide chain
DILLTQSPVILSVSPGERVSFSCRASQSIGTNIHWYQQRTNGSPRLLIKYASESISGIPSRFSGSGSGTDFTLSINSVESEDIADYYCQQNNNWPTTFGAGTKLELKGGGGSGGGGSGGGGSGGGGSQVQLKQSGPGLVQPSQSLSITCTVSGFSLTNYGVHWVRQSPGKGLEWLGVIWSGGNTDYNTPFTSRLSINKDNSKSQVFFKMNSLQSNDTAIYYCARALTYYDYEFAYWGQGTLVTVSAGGGGSGGGGSGGGGSQVQLQQSGGGLVKPSQSLSLTCTVSGFSLTSYGVHWVRQPPGKGLEWIGLIWSGGGTDYNPSLKSRLTISRDTSKNQVSFKISSLTAADTAVYYCARQLGLRAMDYWGQGTSVTVSSASTKGPSVFPLAPSSKSTSGGTAALGCLVKDYFPEPVTVSWNSGALTSGVHTFPAVLQSSGLYSLSSVVTVPSSSLGTQTYICNVNHKPSNTKVDKKVEPKSCDKTHTCPPCPAPELLGGPSVFLFPPKPKDTLMISRTPEVTCVVVDVSHEDPEVKFNWYVDGVEVHNAKTKPREEQYNSTYRVVSVLTVLHQDWLNGKEYKCKVSNKALPAPIEKTISKAKGQPREPQVYTLPPSREEMTKNQVSLTCLVKGFYPSDIAVEWESNGQPENNYKTTPPVLDSDGSFFLYSKLTVDKSRWQQGNVFSCSVMHEALHNHYTQKSLSLSPGK